European Patent Specification EP 3 805 408 B1, published June 21, 2023. Title: Method for Detecting Target Nucleic Acid Using Rolling Circle Amplification and Composition for Detecting Target Nucleic Acid. Applicant: Korea University Research and Business Foundation. The sequence listing filed with the application follows.

SEQUENCE LISTING (8 sequences)

SEQ ID NO: 1 - DNA, 96 bp, Artificial Sequence
  Template_1
tagtgatttcaccccgcatgctagtatcgacgtccccaacatcagtcagctgctgataagctgaaagcaacaaggataggggccccctctcctgct

SEQ ID NO: 2 - DNA, 50 bp, Artificial Sequence
  Wild type
cgagatcctctctctgaaatcactgagcaggagaaagattttctatggag

SEQ ID NO: 3 - DNA, 50 bp, Artificial Sequence
  Mutant
cgagatcctctctctgaaatcactaagcaggagaaagattttctatggag

SEQ ID NO: 4 - DNA, 21 bp, Artificial Sequence
  primer
gggacgtcgatactagcatgc

SEQ ID NO: 5 - DNA, 38 bp, Artificial Sequence
  cutting DNA
gcgcgtcaacatcagtcagctgctgataagctacgcgc

SEQ ID NO: 6 - DNA, 98 bp, Artificial Sequence
  Template_2
agtgatttcacccccatgtagtagtatcgacgtccccccccgtataccccccgtttcctcatatccagtttccccccgtatacccccctctcctgctt

SEQ ID NO: 7 - DNA, 21 bp, Artificial Sequence
  primer
gggacgtcgatactactacat

SEQ ID NO: 8 - DNA, 15 bp, Artificial Sequence
  cutting DNA
cccgtataccccggg